European Patent Application EP 4 640 847 A2, published October 29, 2025. Title: METHOD FOR PREFERENTIALLY AMPLIFYING NUCLEIC ACID MOLECULES LONGER THAN 1 KBP. Applicant: Illumina Singapore Pte. Ltd. Application EP. The sequence listing filed with the application follows.

SEQUENCE LISTING (136 sequences)

SEQ ID NO: 1 - DNA, 2325 bp, synthetic construct
  misc_feature 1..2325: note = DNA polymerase from Thermococcus sp. KS-1
  source 1..2325: mol_type = other DNA
atgatcctcgacactgactacataactgagaatggaaaacccgtcataaggattttcaagaaggagaacggcgagtttaagattgagtacgataggacttttgaaccctacatttacgccctcctgaaggacgattctgccattgaggaggtcaagaagataaccgccgagaggcacggaacggttgtaacggttaagcgggctgaaaaggttcagaagaagttcctcgggagaccagttgaggtctggaaactctactttactcaccctcaggacgtcccagcgataagggacaagatacgagagcatccagcagttattgacatctacgagtacgacatacccttcgccaagcgctacctcatagacaagggattagtgccaatggaaggcgacgaggagctgaaaatgcttgcctttgatatcgagacgctctaccatgagggcgaggagttcgccgaggggccaatccttatgataagctacgccgacgaggaaggggccagggtgataacgtggaagaacgcggatctgccctacgttgacgtcgtctcgacggagagggagatgataaagcgcttcctaaaggtggtcaaagagaaagatcctgacgtcctaataacctacaacggcgacaacttcgacttcgcctacctaaaaaaacgctgtgaaaagcttggaataaacttcacgctcggaagggacggaagcgagccgaagattcagaggatgggcgacaggtttgccgtcgaagtgaagggacggatacacttcgatctctatcctgtgataagacggacgataaacctgcccacatacacgcttgaggccgtttatgaagccgtcttcggtcagccgaaggagaaggtctacgctgaggagatagctacagcttgggagagcggtgaaggccttgagagagtagccagatactcgatggaagatgcgaaggtcacatacgagcttgggaaggagtttttccctatggaggcccagctttctcgcttaatcggccagtccctctgggacgtctcccgctccagcactggcaacctcgttgagtggttcctcctcaggaaggcctacgagaggaatgagctggccccgaacaagcccgatgaaaaggagctggccagaagacgacagagctatgaaggaggctatgtaaaagagcccgagagagggttgtgggagaacatagtgtacctagattttagatctctgtacccctcaatcatcatcacccacaacgtctcgccggatactctcaacagggaaggatgcaaggaatatgacgttgccccccaggtcggtcaccgcttctgcaaggacttcccaggatttatcccgagcctgcttggagacctcctagaggagaggcagaagataaagaagaagatgaaggccacgattgacccgatcgagaggaagctcctcgattacaggcagagggccatcaagatcctggccaacagctactacggttactacggctatgcaagggcgcgctggtactgcaaggagtgtgcagagagcgtaacggcctggggaagggagtacataacgatgaccatcagagagatagaggaaaagtacggctttaaggtaatctacagcgacaccgacggattttttgccacaatacctggagccgatgctgaaaccgtcaaaaagaaggcgatggagttcctcaagtatatcaacgccaaactcccgggcgcgcttgagctcgagtacgagggcttctacaaacgcggcttcttcgtcacgaagaagaagtacgcggtgatagacgaggaaggcaagataacaacgcgcggacttgagattgtgaggcgcgactggagcgagatagcgaaagagacgcaggcgagggttcttgaagctttgctaaaggacggtgacgtcgagaaggccgtgaggatagtcaaagaagttaccgaaaagctgagcaagtacgaggttccgccggagaagctggtgatccacgagcagataacgagggatttaaaggactacaaggcaaccggtccccacgttgccgttgccaagaggttggccgcgagaggagtcaaaatacgccctggaacggtgataagctacatcgtgctcaagggctctgggaggataggcgacagggcgataccgttcgacgagttcgacccgacgaagcacaagtacgacgccgagtactacattgagaaccaggttctcccagccgttgagagaattctgagagccttcggttaccgcaaggaagacctgcgctaccagaagacgagacaggttggtctgggagcctggctgaagccgaagggaacttga

SEQ ID NO: 2 - protein, 774 aa, synthetic construct
  REGION 1..774: note = DNA polymerase from Thermococcus sp. KS-1
MILDTDYITENGKPVIRIFKKENGEFKIEYDRTFEPYIYALLKDDSAIEEVKKITAERHGTVVTVKRAEKVQKKFLGRPVEVWKLYFTHPQDVPAIRDKIREHPAVIDIYEYDIPFAKRYLIDKGLVPMEGDEELKMLAFDIETLYHEGEEFAEGPILMISYADEEGARVITWKNADLPYVDVVSTEREMIKRFLKVVKEKDPDVLITYNGDNFDFAYLKKRCEKLGINFTLGRDGSEPKIQRMGDRFAVEVKGRIHFDLYPVIRRTINLPTYTLEAVYEAVFGQPKEKVYAEEIATAWESGEGLERVARYSMEDAKVTYELGKEFFPMEAQLSRLIGQSLWDVSRSSTGNLVEWFLLRKAYERNELAPNKPDEKELARRRQSYEGGYVKEPERGLWENIVYLDFRSLYPSIIITHNVSPDTLNREGCKEYDVAPQVGHRFCKDFPGFIPSLLGDLLEERQKIKKKMKATIDPIERKLLDYRQRAIKILANSYYGYYGYARARWYCKECAESVTAWGREYITMTIREIEEKYGFKVIYSDTDGFFATIPGADAETVKKKAMEFLKYINAKLPGALELEYEGFYKRGFFVTKKKYAVIDEEGKITTRGLEIVRRDWSEIAKETQARVLEALLKDGDVEKAVRIVKEVTEKLSKYEVPPEKLVIHEQITRDLKDYKATGPHVAVAKRLAARGVKIRPGTVISYIVLKGSGRIGDRAIPFDEFDPTKHKYDAEYYIENQVLPAVERILRAFGYRKEDLRYQKTRQVGLGAWLKPKGT

SEQ ID NO: 3 - DNA, 2325 bp, synthetic construct
  misc_feature 1..2325: note = DNA polymerase from Thermococcus celer
  source 1..2325: mol_type = other DNA
atgatcctcgacgctgactacatcaccgaagatgggaagcccgtcgtgaggatattcaggaaggagaagggcgagttcagaatcgactacgacagggacttcgagccctacatctacgccctcctgaaggacgattcggccatcgaggaggtgaagaggataaccgttgagcgccacgggaaggccgtcagggttaagcgggtggagaaggtcgaaaagaagttcctcaacaggccgatagaggtctggaagctctacttcaatcacccgcaggacgttccggcgataagggacgagataaggaagcatccggccgtcgttgatatctacgagtacgacatccccttcgccaagcgctacctcatcgataaggggctcgtcccgatggagggggaggaggagctcaaactgatggccttcgacatcgagaccctctaccacgagggagacgagttcggggaggggccgatcctgatgataagctacgccgacggggacggggcgagggtcataacctggaagaagatcgacctcccctacgtcgacgtcgtctcgaccgagaaggagatgataaagcgcttcctccaggtggtgaaggagaaggacccggacgtgctcgtaacttacaacggcgacaacttcgacttcgcctacctgaagagacgctccgaggagcttggattgaagttcatcctcgggagggacgggagcgagcccaagatccagcgcatgggcgaccgcttcgccgtcgaggtgaaggggaggatacacttcgacctctacccggtgataaggcgcaccgtgaacctgccgacctacacgctcgaggcggtctacgaggccatcttcgggaggccaaaggagaaggtctacgccggggagatagtggaggcctgggaaaccggcgagggtcttgagagggttgcccgctactccatggaggacgcaaaggttaccttcgagctcgggagggagttcttcccgatggaggcccagctctcgaggctcatcggccagggtctctgggacgtctcccgctcgagcaccggcaacctggtcgagtggttcctcctgaggaaggcctacgagaggaacgaactggccccgaacaagccgagcggccgggaagtggagatcaggaggcgtggctacgccggtggttacgttaaggagccggagaggggtttatgggagaacatcgtgtacctcgactttcgctctctttacccctccatcatcataacccacaacgtctcgcccgataccctaaacagggagggctgtgagaactacgacgtcgccccccaggtggggcataagttctgcaaagattttccgggcttcatcccgagcctgctcggaggcctgcttgaggagaggcagaagataaagcggaggatgaaggcctctgtggatcccgttgagcggaagctcctcgattacaggcagagggccatcaagatactggccaacagcttctacggatactacggctacgcgagggcgaggtggtactgcagggagtgcgcggagagcgttaccgcctggggcagggagtacatcgatagggtcatcagggagctcgaggagaagttcggcttcaaggtgctctacgcggacacggacggactgcacgccacgatccccggggcggacgccgggaccgtcaaggagagggcgagggggttcctgagatacatcaaccccaagctccccggcctcctggagctcgagtacgaggggttctacctgaggggtttcttcgtgacgaagaagaagtacgcggtcatagacgaggagggcaagataaccacgcgcggcctcgagatagtcaggcgggactggagcgaggtggccaaggagacgcaggcgagggtcctggaggcgatactgaggcacggtgacgtcgaggaggccgttagaatcgtcagggaggtaaccgaaaagctgagcaagtacgaggttccgccggagaaactggtgatccacgagcagataacgagggatttgagggactacaaagccacgggaccgcacgtggcggtggcgaagcgcctggccgggaggggggtaaggatacgccccgggacggtgataagctacatcgtcctcaagggctccggaaggataggggacagggcgattcccttcgacgagttcgacccgactaagcacaggtacgacgccgactactacatcgagaaccaggttctgccagccgtcgagaggatcctgaaggccttcggctaccgcaaggaggacctgaaataccagaagacgaggcaggtgggcctgggtgcgtggctcaacgcggggaaggggtga

SEQ ID NO: 4 - protein, 774 aa, synthetic construct
  REGION 1..774: note = DNA polymerase from Thermococcus celer
MILDADYITEDGKPVVRIFRKEKGEFRIDYDRDFEPYIYALLKDDSAIEEVKRITVERHGKAVRVKRVEKVEKKFLNRPIEVWKLYFNHPQDVPAIRDEIRKHPAVVDIYEYDIPFAKRYLIDKGLVPMEGEEELKLMAFDIETLYHEGDEFGEGPILMISYADGDGARVITWKKIDLPYVDVVSTEKEMIKRFLQVVKEKDPDVLVTYNGDNFDFAYLKRRSEELGLKFILGRDGSEPKIQRMGDRFAVEVKGRIHFDLYPVIRRTVNLPTYTLEAVYEAIFGRPKEKVYAGEIVEAWETGEGLERVARYSMEDAKVTFELGREFFPMEAQLSRLIGQGLWDVSRSSTGNLVEWFLLRKAYERNELAPNKPSGREVEIRRRGYAGGYVKEPERGLWENIVYLDFRSLYPSIIITHNVSPDTLNREGCENYDVAPQVGHKFCKDFPGFIPSLLGGLLEERQKIKRRMKASVDPVERKLLDYRQRAIKILANSFYGYYGYARARWYCRECAESVTAWGREYIDRVIRELEEKFGFKVLYADTDGLHATIPGADAGTVKERARGFLRYINPKLPGLLELEYEGFYLRGFFVTKKKYAVIDEEGKITTRGLEIVRRDWSEVAKETQARVLEAILRHGDVEEAVRIVREVTEKLSKYEVPPEKLVIHEQITRDLRDYKATGPHVAVAKRLAGRGVRIRPGTVISYIVLKGSGRIGDRAIPFDEFDPTKHRYDADYYIENQVLPAVERILKAFGYRKEDLKYQKTRQVGLGAWLNAGKG

SEQ ID NO: 5 - DNA, 2328 bp, synthetic construct
  misc_feature 1..2328: note = DNA polymerase from Thermococcus siculi
  source 1..2328: mol_type = other DNA
atgatcctcgacacggactacatcacggaagatgggaaacccgtcataaggatattcaagaaagagaacggcgagttcaagatcgagtacgacaggacttttgaaccctacatctacgccctcctgaaggacgactccgcgattgaggatgttaaaaagataaccgccgagaggcacggaacggtggtgaaggtcaagcgcgccgaaaaggtgcagaagaagttcctaggcaggccggttgaagtctggaagctctacttcacccacccccaagatgtcccggcgataagggacaagattaggaagcatccagctgtaattgacatctacgagtacgacataccattcgccaagcgctacctcatcgacaagggcctgattccgatggagggtgaagaagagcttaagatgctcgccttcgacattgagacgctctaccatgagggtgaggagttcgccgaggggcctattctgatgataagctacgccgacgagagcgaggcacgcgtcatcacctggaagaaaatcgacctcccctacgttgacgtcgtctcaacggagaaggagatgataaagcgcttcctccgcgttgtgaaggagaaagatcccgatgtcctcataacctacaacggcgacaacttcgacttcgcctacctgaagaagcgctgtgaaaagcttggaataaacttcctccttggaagggacgggagcgagccgaagatccagagaatgggtgaccgcttcgccgttgaggtgaaggggaggatacacttcgacctctatcctgtaataaggcgcacgataaacctgccgacctacatgcttgaggcagtctacgaggccatctttgggaagccaaaggagaaggtttacgccgaggagatagccaccgcttgggaaaccggagagggccttgagagggtggctcgctactctatggaggacgcgaaggtcacgtttgagcttggaaaggagttcttcccgatggaggcccaactttcgaggttggtcggccagagcttctgggatgtcgcgcgctcaagcacgggcaatctggtcgagtggttcctcctcaggaaggcctacgagaggaacgagctggctccaaacaagccctctggaagggaatatgacgagaggcgcggtggatacgccggcggctacgtcaaggaaccggaaaagggcctgtgggagaacatagtctacctcgactataaatctctctacccctcaatcatcatcacccacaacgtctcgcccgataccctcaaccgcgagggctgtaaggagtatgacgtagctccacaggtcggccaccgcttctgcaaggactttccaggcttcatcccgagcctgctcggggatctcctggaggagaggcagaagataaagaggaagatgaaggcaacaattgacccgatcgagagaaagctccttgattacaggcaacgggccatcaagatccttctaaatagtttttacggctactacggctacgcaagggctcgctggtactgcaaggagtgtgccgagagcgttacggcatggggaagggaatatatcaccatgacaatcagggaaatagaagagaagtatggctttaaagtactttatgcggacactgacggcttcttcgcgacgattcccggggaagatgccgagaccatcaaaaagagggcgatggagttcctcaagtacataaacgccaaactccccggtgcgctcgaacttgagtacgaggacttctacaggcgcggcttcttcgtcaccaagaagaaatacgcggttatcgacgaggagggcaagataacaacgcgcgggctggagatcgtcaggcgcgactggagcgagatagccaaggagacgcaggcgcgggttctggaggcccttctgaaggacggtgacgtcgaagaggccgtgagcatagtcaaagaagtgaccgagaagctgagcaagtacgaggttccgccggagaagctcgttatccacgagcagataacgcgcgagctgaaggactacaaggcaacgggaccacacgtggcgatagcgaagaggttagccgcgagaggcgtcaaaatccgccccgggacagtcatcagctacatcgtgctcaagggctccgggaggataggcgacagggcgattcccttcgacgagttcgaccccacgaagcacaagtacgatgcagagtactacatcgagaaccaggttctacctgccgtcgagaggattctgaaggccttcggctatcgcggtgaggagctcagataccagaagacgaggcaggttggacttggggcgtggctgaagccgaaggggaaggggtga

SEQ ID NO: 6 - protein, 775 aa, synthetic construct
  REGION 1..775: note = DNA polymerase from Thermococcus siculi
MILDTDYITEDGKPVIRIFKKENGEFKIEYDRTFEPYIYALLKDDSAIEDVKKITAERHGTVVKVKRAEKVQKKFLGRPVEVWKLYFTHPQDVPAIRDKIRKHPAVIDIYEYDIPFAKRYLIDKGLIPMEGEEELKMLAFDIETLYHEGEEFAEGPILMISYADESEARVITWKKIDLPYVDVVSTEKEMIKRFLRVVKEKDPDVLITYNGDNFDFAYLKKRCEKLGINFLLGRDGSEPKIQRMGDRFAVEVKGRIHFDLYPVIRRTINLPTYMLEAVYEAIFGKPKEKVYAEEIATAWETGEGLERVARYSMEDAKVTFELGKEFFPMEAQLSRLVGQSFWDVARSSTGNLVEWFLLRKAYERNELAPNKPSGREYDERRGGYAGGYVKEPEKGLWENIVYLDYKSLYPSIIITHNVSPDTLNREGCKEYDVAPQVGHRFCKDFPGFIPSLLGDLLEERQKIKRKMKATIDPIERKLLDYRQRAIKILLNSFYGYYGYARARWYCKECAESVTAWGREYITMTIREIEEKYGFKVLYADTDGFFATIPGEDAETIKKRAMEFLKYINAKLPGALELEYEDFYRRGFFVTKKKYAVIDEEGKITTRGLEIVRRDWSEIAKETQARVLEALLKDGDVEEAVSIVKEVTEKLSKYEVPPEKLVIHEQITRELKDYKATGPHVAIAKRLAARGVKIRPGTVISYIVLKGSGRIGDRAIPFDEFDPTKHKYDAEYYIENQVLPAVERILKAFGYRGEELRYQKTRQVGLGAWLKPKGKG

SEQ ID NO: 7 - protein, 774 aa, synthetic construct
  REGION 1..774: note = DNA polymerase from Thermococcus kodakarensis
MILDTDYITEDGKPVIRIFKKENGEFKIEYDRTFEPYFYALLKDDSAIEEVKKITAERHGTVVTVKRVEKVQKKFLGRPVEVWKLYFTHPQDVPAIRDKIREHPAVIDIYEYDIPFAKRYLIDKGLVPMEGDEELKMLAFDIETLYEEGEEFAEGPILMISYADEEGARVITWKNVDLPYVDVVSTEREMIKRFLRVVKEKDPDVLITYNGDNFDFAYLKKRCEKLGINFALGRDGSEPKIQRMGDRFAVEVKGRIHFDLYPVIRRTINLPTYTLEAVYEAVFGQPKEKVYAEEITTAWETGENLERVARYSMEDAKVTYELGKEFLPMEAQLSRLIGQSLWDVSRSSTGNLVEWFLLRKAYERNELAPNKPDEKELARRRQSYEGGYVKEPERGLWENIVYLDFRSLYPSIIITHNVSPDTLNREGCKEYDVAPQVGHRFCKDFPGFIPSLLGDLLEERQKIKKKMKATIDPIERKLLDYRQRAIKILANSYYGYYGYARARWYCKECAESVTAWGREYITMTIKEIEEKYGFKVIYSDTDGFFATIPGADAETVKKKAMEFLKYINAKLPGALELEYEGFYERGFFVTKKKYAVIDEEGKITTRGLEIVRRDWSEIAKETQARVLEALLKDGDVEKAVRIVKEVTEKLSKYEVPPEKLVIHEQITRDLKDYKATGPHVAVAKRLAARGVKIRPGTVISYIVLKGSGRIGDRAIPFDEFDPTKHKYDAEYYIENQVLPAVERILRAFGYRKEDLRYQKTRQVGLSAWLKPKGT

SEQ ID NO: 8 - DNA, 13 bp, synthetic construct
  misc_feature 1..13: note = Sample tag sequence
  source 1..13: mol_type = other DNA
tagaattgaagaa

SEQ ID NO: 9 - DNA, 13 bp, synthetic construct
  misc_feature 1..13: note = Sample tag sequence
  source 1..13: mol_type = other DNA
tggccatagctac

SEQ ID NO: 10 - DNA, 13 bp, synthetic construct
  misc_feature 1..13: note = Sample tag sequence
  source 1..13: mol_type = other DNA
gtcatctgcgacc

SEQ ID NO: 11 - DNA, 13 bp, synthetic construct
  misc_feature 1..13: note = Sample tag sequence
  source 1..13: mol_type = other DNA
ttcgcgcttggac

SEQ ID NO: 12 - DNA, 13 bp, synthetic construct
  misc_feature 1..13: note = Sample tag sequence
  source 1..13: mol_type = other DNA
cgcgaaccgttag

SEQ ID NO: 13 - DNA, 13 bp, synthetic construct
  misc_feature 1..13: note = Sample tag sequence
  source 1..13: mol_type = other DNA
ttgcagcctctaa

SEQ ID NO: 14 - DNA, 13 bp, synthetic construct
  misc_feature 1..13: note = Sample tag sequence
  source 1..13: mol_type = other DNA
tctactagtacga

SEQ ID NO: 15 - DNA, 13 bp, synthetic construct
  misc_feature 1..13: note = Sample tag sequence
  source 1..13: mol_type = other DNA
gtaggttctactg

SEQ ID NO: 16 - DNA, 13 bp, synthetic construct
  misc_feature 1..13: note = Sample tag sequence
  source 1..13: mol_type = other DNA
gccaatatcaagt

SEQ ID NO: 17 - DNA, 13 bp, synthetic construct
  misc_feature 1..13: note = Sample tag sequence
  source 1..13: mol_type = other DNA
ctatcttgctggt

SEQ ID NO: 18 - DNA, 13 bp, synthetic construct
  misc_feature 1..13: note = Sample tag sequence
  source 1..13: mol_type = other DNA
gttctcataggta

SEQ ID NO: 19 - DNA, 13 bp, synthetic construct
  misc_feature 1..13: note = Sample tag sequence
  source 1..13: mol_type = other DNA
gtctatgaaccaa

SEQ ID NO: 20 - DNA, 13 bp, synthetic construct
  misc_feature 1..13: note = Sample tag sequence
  source 1..13: mol_type = other DNA
cggagcgcttatt

SEQ ID NO: 21 - DNA, 13 bp, synthetic construct
  misc_feature 1..13: note = Sample tag sequence
  source 1..13: mol_type = other DNA
tatgccatgagga

SEQ ID NO: 22 - DNA, 13 bp, synthetic construct
  misc_feature 1..13: note = Sample tag sequence
  source 1..13: mol_type = other DNA
atacgactcggag

SEQ ID NO: 23 - DNA, 13 bp, synthetic construct
  misc_feature 1..13: note = Sample tag sequence
  source 1..13: mol_type = other DNA
gatggaactcagc

SEQ ID NO: 24 - DNA, 13 bp, synthetic construct
  misc_feature 1..13: note = Sample tag sequence
  source 1..13: mol_type = other DNA
ggacctgcatgaa

SEQ ID NO: 25 - DNA, 13 bp, synthetic construct
  misc_feature 1..13: note = Sample tag sequence
  source 1..13: mol_type = other DNA
tagactggaactt

SEQ ID NO: 26 - DNA, 13 bp, synthetic construct
  misc_feature 1..13: note = Sample tag sequence
  source 1..13: mol_type = other DNA
gaattacctcgtt

SEQ ID NO: 27 - DNA, 13 bp, synthetic construct
  misc_feature 1..13: note = Sample tag sequence
  source 1..13: mol_type = other DNA
aggatcaggctac

SEQ ID NO: 28 - DNA, 13 bp, synthetic construct
  misc_feature 1..13: note = Sample tag sequence
  source 1..13: mol_type = other DNA
acgcgtagaagag

SEQ ID NO: 29 - DNA, 13 bp, synthetic construct
  misc_feature 1..13: note = Sample tag sequence
  source 1..13: mol_type = other DNA
cttcgagacttac

SEQ ID NO: 30 - DNA, 13 bp, synthetic construct
  misc_feature 1..13: note = Sample tag sequence
  source 1..13: mol_type = other DNA
gacggctaactcc

SEQ ID NO: 31 - DNA, 13 bp, synthetic construct
  misc_feature 1..13: note = Sample tag sequence
  source 1..13: mol_type = other DNA
ttagcattctctt

SEQ ID NO: 32 - DNA, 13 bp, synthetic construct
  misc_feature 1..13: note = Sample tag sequence
  source 1..13: mol_type = other DNA
gcaaggcatagta

SEQ ID NO: 33 - DNA, 13 bp, synthetic construct
  misc_feature 1..13: note = Sample tag sequence
  source 1..13: mol_type = other DNA
acctagatatgga

SEQ ID NO: 34 - DNA, 13 bp, synthetic construct
  misc_feature 1..13: note = Sample tag sequence
  source 1..13: mol_type = other DNA
acgccaaggcgta

SEQ ID NO: 35 - DNA, 13 bp, synthetic construct
  misc_feature 1..13: note = Sample tag sequence
  source 1..13: mol_type = other DNA
tatgacggatccg

SEQ ID NO: 36 - DNA, 13 bp, synthetic construct
  misc_feature 1..13: note = Sample tag sequence
  source 1..13: mol_type = other DNA
cctccattagaga

SEQ ID NO: 37 - DNA, 13 bp, synthetic construct
  misc_feature 1..13: note = Sample tag sequence
  source 1..13: mol_type = other DNA
attgaatactctg

SEQ ID NO: 38 - DNA, 13 bp, synthetic construct
  misc_feature 1..13: note = Sample tag sequence
  source 1..13: mol_type = other DNA
gagatgagaagaa

SEQ ID NO: 39 - DNA, 13 bp, synthetic construct
  misc_feature 1..13: note = Sample tag sequence
  source 1..13: mol_type = other DNA
tctgagtagccgg

SEQ ID NO: 40 - DNA, 13 bp, synthetic construct
  misc_feature 1..13: note = Sample tag sequence
  source 1..13: mol_type = other DNA
aataggtagtacg

SEQ ID NO: 41 - DNA, 13 bp, synthetic construct
  misc_feature 1..13: note = Sample tag sequence
  source 1..13: mol_type = other DNA
gtcgaagaagtcc

SEQ ID NO: 42 - DNA, 13 bp, synthetic construct
  misc_feature 1..13: note = Sample tag sequence
  source 1..13: mol_type = other DNA
tactgcatctcgt

SEQ ID NO: 43 - DNA, 13 bp, synthetic construct
  misc_feature 1..13: note = Sample tag sequence
  source 1..13: mol_type = other DNA
gacgtattagagc

SEQ ID NO: 44 - DNA, 13 bp, synthetic construct
  misc_feature 1..13: note = Sample tag sequence
  source 1..13: mol_type = other DNA
cctgcattattcg

SEQ ID NO: 45 - DNA, 13 bp, synthetic construct
  misc_feature 1..13: note = Sample tag sequence
  source 1..13: mol_type = other DNA
acgaatgatgctc

SEQ ID NO: 46 - DNA, 13 bp, synthetic construct
  misc_feature 1..13: note = Sample tag sequence
  source 1..13: mol_type = other DNA
tactagcagagat

SEQ ID NO: 47 - DNA, 13 bp, synthetic construct
  misc_feature 1..13: note = Sample tag sequence
  source 1..13: mol_type = other DNA
ctcctcatcttcc

SEQ ID NO: 48 - DNA, 13 bp, synthetic construct
  misc_feature 1..13: note = Sample tag sequence
  source 1..13: mol_type = other DNA
tcctctgcgctgc

SEQ ID NO: 49 - DNA, 13 bp, synthetic construct
  misc_feature 1..13: note = Sample tag sequence
  source 1..13: mol_type = other DNA
ccttctcagtccg

SEQ ID NO: 50 - DNA, 13 bp, synthetic construct
  misc_feature 1..13: note = Sample tag sequence
  source 1..13: mol_type = other DNA
cagcttcatagcg

SEQ ID NO: 51 - DNA, 13 bp, synthetic construct
  misc_feature 1..13: note = Sample tag sequence
  source 1..13: mol_type = other DNA
ttgactctcgcgc

SEQ ID NO: 52 - DNA, 13 bp, synthetic construct
  misc_feature 1..13: note = Sample tag sequence
  source 1..13: mol_type = other DNA
tatcctgagcgat

SEQ ID NO: 53 - DNA, 13 bp, synthetic construct
  misc_feature 1..13: note = Sample tag sequence
  source 1..13: mol_type = other DNA
aacgcctagccga

SEQ ID NO: 54 - DNA, 13 bp, synthetic construct
  misc_feature 1..13: note = Sample tag sequence
  source 1..13: mol_type = other DNA
ccgaagacgtcat

SEQ ID NO: 55 - DNA, 13 bp, synthetic construct
  misc_feature 1..13: note = Sample tag sequence
  source 1..13: mol_type = other DNA
gagttctccagat

SEQ ID NO: 56 - DNA, 13 bp, synthetic construct
  misc_feature 1..13: note = Sample tag sequence
  source 1..13: mol_type = other DNA
tgcatccgcgctt

SEQ ID NO: 57 - DNA, 13 bp, synthetic construct
  misc_feature 1..13: note = Sample tag sequence
  source 1..13: mol_type = other DNA
cctgaactcaagt

SEQ ID NO: 58 - DNA, 13 bp, synthetic construct
  misc_feature 1..13: note = sample tag sequence
  source 1..13: mol_type = other DNA
ggtcgtatgcgta

SEQ ID NO: 59 - DNA, 13 bp, synthetic construct
  misc_feature 1..13: note = Sample tag sequence
  source 1..13: mol_type = other DNA
aggcctctctacc

SEQ ID NO: 60 - DNA, 13 bp, synthetic construct
  misc_feature 1..13: note = Sample tag sequence
  source 1..13: mol_type = other DNA
gtactccatccaa

SEQ ID NO: 61 - DNA, 13 bp, synthetic construct
  misc_feature 1..13: note = Sample tag sequence
  source 1..13: mol_type = other DNA
cagcggacgcgct

SEQ ID NO: 62 - DNA, 13 bp, synthetic construct
  misc_feature 1..13: note = Sample tag sequence
  source 1..13: mol_type = other DNA
atctctcttagca

SEQ ID NO: 63 - DNA, 13 bp, synthetic construct
  misc_feature 1..13: note = Sample tag sequence
  source 1..13: mol_type = other DNA
aagcaataataat

SEQ ID NO: 64 - DNA, 13 bp, synthetic construct
  misc_feature 1..13: note = Sample tag sequence
  source 1..13: mol_type = other DNA
aaggcgactccga

SEQ ID NO: 65 - DNA, 13 bp, synthetic construct
  misc_feature 1..13: note = Sample tag sequence
  source 1..13: mol_type = other DNA
acgtctctaggag

SEQ ID NO: 66 - DNA, 13 bp, synthetic construct
  misc_feature 1..13: note = Sample tag sequence
  source 1..13: mol_type = other DNA
ccatcagacctct

SEQ ID NO: 67 - DNA, 13 bp, synthetic construct
  misc_feature 1..13: note = Sample tag sequence
  source 1..13: mol_type = other DNA
acttaatcgtact

SEQ ID NO: 68 - DNA, 13 bp, synthetic construct
  misc_feature 1..13: note = Sample tag sequence
  source 1..13: mol_type = other DNA
tggaattctccaa

SEQ ID NO: 69 - DNA, 13 bp, synthetic construct
  misc_feature 1..13: note = Sample tag sequence
  source 1..13: mol_type = other DNA
ccatacgatcagg

SEQ ID NO: 70 - DNA, 13 bp, synthetic construct
  misc_feature 1..13: note = Sample tag sequence
  source 1..13: mol_type = other DNA
ttatggagcaata

SEQ ID NO: 71 - DNA, 13 bp, synthetic construct
  misc_feature 1..13: note = Sample tag sequence
  source 1..13: mol_type = other DNA
gctcggcgttcga

SEQ ID NO: 72 - DNA, 13 bp, synthetic construct
  misc_feature 1..13: note = Sample tag sequence
  source 1..13: mol_type = other DNA
ttggccagtcgct

SEQ ID NO: 73 - DNA, 13 bp, synthetic construct
  misc_feature 1..13: note = Sample tag sequence
  source 1..13: mol_type = other DNA
cagatacgtagag

SEQ ID NO: 74 - DNA, 13 bp, synthetic construct
  misc_feature 1..13: note = Sample tag sequence
  source 1..13: mol_type = other DNA
aatgctattatcc

SEQ ID NO: 75 - DNA, 13 bp, synthetic construct
  misc_feature 1..13: note = Sample tag sequence
  source 1..13: mol_type = other DNA
gcagcatgccgat

SEQ ID NO: 76 - DNA, 13 bp, synthetic construct
  misc_feature 1..13: note = Sample tag sequence
  source 1..13: mol_type = other DNA
ggagagttacctc

SEQ ID NO: 77 - DNA, 13 bp, synthetic construct
  misc_feature 1..13: note = Sample tag sequence
  source 1..13: mol_type = other DNA
gagagtccatgat

SEQ ID NO: 78 - DNA, 13 bp, synthetic construct
  misc_feature 1..13: note = Sample tag sequence
  source 1..13: mol_type = other DNA
caatctattctga

SEQ ID NO: 79 - DNA, 13 bp, synthetic construct
  misc_feature 1..13: note = Sample tag sequence
  source 1..13: mol_type = other DNA
gctcttagtatcc

SEQ ID NO: 80 - DNA, 13 bp, synthetic construct
  misc_feature 1..13: note = Sample tag sequence
  source 1..13: mol_type = other DNA
ccatagttatggt

SEQ ID NO: 81 - DNA, 13 bp, synthetic construct
  misc_feature 1..13: note = Sample tag sequence
  source 1..13: mol_type = other DNA
tgcgagatcgaag

SEQ ID NO: 82 - DNA, 13 bp, synthetic construct
  misc_feature 1..13: note = Sample tag sequence
  source 1..13: mol_type = other DNA
agagaagtcgagt

SEQ ID NO: 83 - DNA, 13 bp, synthetic construct
  misc_feature 1..13: note = Sample tag sequence
  source 1..13: mol_type = other DNA
ggtaactccatat

SEQ ID NO: 84 - DNA, 13 bp, synthetic construct
  misc_feature 1..13: note = Sample tag sequence
  source 1..13: mol_type = other DNA
tgctattccaggc

SEQ ID NO: 85 - DNA, 13 bp, synthetic construct
  misc_feature 1..13: note = Sample tag sequence
  source 1..13: mol_type = other DNA
aaccgcgaggctc

SEQ ID NO: 86 - DNA, 13 bp, synthetic construct
  misc_feature 1..13: note = Sample tag sequence
  source 1..13: mol_type = other DNA
ttctagagatacc

SEQ ID NO: 87 - DNA, 13 bp, synthetic construct
  misc_feature 1..13: note = Sample tag sequence
  source 1..13: mol_type = other DNA
ttcgctcaagtat

SEQ ID NO: 88 - DNA, 13 bp, synthetic construct
  misc_feature 1..13: note = Sample tag sequence
  source 1..13: mol_type = other DNA
cagagaaggcgca

SEQ ID NO: 89 - DNA, 13 bp, synthetic construct
  misc_feature 1..13: note = Sample tag sequence
  source 1..13: mol_type = other DNA
tagaattggcctc

SEQ ID NO: 90 - DNA, 13 bp, synthetic construct
  misc_feature 1..13: note = Sample tag sequence
  source 1..13: mol_type = other DNA
ggccattctccag

SEQ ID NO: 91 - DNA, 13 bp, synthetic construct
  misc_feature 1..13: note = Sample tag sequence
  source 1..13: mol_type = other DNA
tccaacgcgcgtt

SEQ ID NO: 92 - DNA, 13 bp, synthetic construct
  misc_feature 1..13: note = Sample tag sequence
  source 1..13: mol_type = other DNA
gccgcagattacg

SEQ ID NO: 93 - DNA, 13 bp, synthetic construct
  misc_feature 1..13: note = Sample tag sequence
  source 1..13: mol_type = other DNA
gcagttcgaacgc

SEQ ID NO: 94 - DNA, 13 bp, synthetic construct
  misc_feature 1..13: note = Sample tag sequence
  source 1..13: mol_type = other DNA
ttctctctgcagg

SEQ ID NO: 95 - DNA, 13 bp, synthetic construct
  misc_feature 1..13: note = Sample tag sequence
  source 1..13: mol_type = other DNA
taagctaccagcg

SEQ ID NO: 96 - DNA, 13 bp, synthetic construct
  misc_feature 1..13: note = Sample tag sequence
  source 1..13: mol_type = other DNA
ctgcatgaggttg

SEQ ID NO: 97 - DNA, 13 bp, synthetic construct
  misc_feature 1..13: note = Sample tag sequence
  source 1..13: mol_type = other DNA
ttgcctagcgagg

SEQ ID NO: 98 - DNA, 13 bp, synthetic construct
  misc_feature 1..13: note = Sample tag sequence
  source 1..13: mol_type = other DNA
caactgaattagg

SEQ ID NO: 99 - DNA, 13 bp, synthetic construct
  misc_feature 1..13: note = Sample tag sequence
  source 1..13: mol_type = other DNA
aagcggtcctctt

SEQ ID NO: 100 - DNA, 13 bp, synthetic construct
  misc_feature 1..13: note = Sample tag sequence
  source 1..13: mol_type = other DNA
aatggaaggaccg

SEQ ID NO: 101 - DNA, 13 bp, synthetic construct
  misc_feature 1..13: note = Sample tag sequence
  source 1..13: mol_type = other DNA
gagttagtaagtt

SEQ ID NO: 102 - DNA, 13 bp, synthetic construct
  misc_feature 1..13: note = Sample tag sequence
  source 1..13: mol_type = other DNA
ttcctaattccaa

SEQ ID NO: 103 - DNA, 13 bp, synthetic construct
  misc_feature 1..13: note = Sample tag sequence
  source 1..13: mol_type = other DNA
gttctggttcgct

SEQ ID NO: 104 - DNA, 13 bp, synthetic construct
  misc_feature 1..13: note = Sample tag sequence
  source 1..13: mol_type = other DNA
gttcatctcttcc

SEQ ID NO: 105 - DNA, 13 bp, synthetic construct
  misc_feature 1..13: note = Sample tag sequence
  source 1..13: mol_type = other DNA
attccgaggaaga

SEQ ID NO: 106 - DNA, 13 bp, synthetic construct
  misc_feature 1..13: note = Sample tag sequence
  source 1..13: mol_type = other DNA
cttagccgagaga

SEQ ID NO: 107 - DNA, 13 bp, synthetic construct
  misc_feature 1..13: note = Sample tag sequence
  source 1..13: mol_type = other DNA
gtctgctacgctt

SEQ ID NO: 108 - DNA, 13 bp, synthetic construct
  misc_feature 1..13: note = Sample tag sequence
  source 1..13: mol_type = other DNA
atggcgccgcgca

SEQ ID NO: 109 - DNA, 13 bp, synthetic construct
  misc_feature 1..13: note = Sample tag sequence
  source 1..13: mol_type = other DNA
taattggttatct

SEQ ID NO: 110 - DNA, 13 bp, synthetic construct
  misc_feature 1..13: note = Sample tag sequence
  source 1..13: mol_type = other DNA
tcggttataagtc

SEQ ID NO: 111 - DNA, 13 bp, synthetic construct
  misc_feature 1..13: note = Sample tag sequence
  source 1..13: mol_type = other DNA
tgcctgagaacgt

SEQ ID NO: 112 - DNA, 13 bp, synthetic construct
  misc_feature 1..13: note = Sample tag sequence
  source 1..13: mol_type = other DNA
agatgcggttaac

SEQ ID NO: 113 - DNA, 13 bp, synthetic construct
  misc_feature 1..13: note = Sample tag sequence
  source 1..13: mol_type = other DNA
atggaataggcga

SEQ ID NO: 114 - DNA, 13 bp, synthetic construct
  misc_feature 1..13: note = Sample tag sequence
  source 1..13: mol_type = other DNA
agagatgcgatcg

SEQ ID NO: 115 - DNA, 13 bp, synthetic construct
  misc_feature 1..13: note = Sample tag sequence
  source 1..13: mol_type = other DNA
ctccaactaacgt

SEQ ID NO: 116 - DNA, 13 bp, synthetic construct
  misc_feature 1..13: note = Sample tag sequence
  source 1..13: mol_type = other DNA
gccttgctactgg

SEQ ID NO: 117 - DNA, 13 bp, synthetic construct
  misc_feature 1..13: note = Sample tag sequence
  source 1..13: mol_type = other DNA
cttcgtctctacg

SEQ ID NO: 118 - DNA, 13 bp, synthetic construct
  misc_feature 1..13: note = Sample tag sequence
  source 1..13: mol_type = other DNA
acgctcatagcct

SEQ ID NO: 119 - DNA, 13 bp, synthetic construct
  misc_feature 1..13: note = Sample tag sequence
  source 1..13: mol_type = other DNA
gtcgaagataagg

SEQ ID NO: 120 - DNA, 13 bp, synthetic construct
  misc_feature 1..13: note = Sample tag sequence
  source 1..13: mol_type = other DNA
gccggagtcctcg

SEQ ID NO: 121 - DNA, 13 bp, synthetic construct
  misc_feature 1..13: note = Sample tag sequence
  source 1..13: mol_type = other DNA
tatacggcgacct

SEQ ID NO: 122 - DNA, 13 bp, synthetic construct
  misc_feature 1..13: note = Sample tag sequence
  source 1..13: mol_type = other DNA
aggtagatattcg

SEQ ID NO: 123 - DNA, 13 bp, synthetic construct
  misc_feature 1..13: note = Sample tag sequence
  source 1..13: mol_type = other DNA
ttaaggtactgct

SEQ ID NO: 124 - DNA, 13 bp, synthetic construct
  misc_feature 1..13: note = Sample tag sequence
  source 1..13: mol_type = other DNA
cggatctggtata

SEQ ID NO: 125 - DNA, 13 bp, synthetic construct
  misc_feature 1..13: note = Sample tag sequence
  source 1..13: mol_type = other DNA
gaggtctcggagg

SEQ ID NO: 126 - DNA, 13 bp, synthetic construct
  misc_feature 1..13: note = Sample tag sequence
  source 1..13: mol_type = other DNA
ggcatcgatggac

SEQ ID NO: 127 - DNA, 13 bp, synthetic construct
  misc_feature 1..13: note = Sample tag sequence
  source 1..13: mol_type = other DNA
gatctccgatata

SEQ ID NO: 128 - DNA, 13 bp, synthetic construct
  misc_feature 1..13: note = Sample tag sequence
  source 1..13: mol_type = other DNA
gattcggaatact

SEQ ID NO: 129 - DNA, 13 bp, synthetic construct
  misc_feature 1..13: note = Sample tag sequence
  source 1..13: mol_type = other DNA
ctgcgatccggcc

SEQ ID NO: 130 - DNA, 13 bp, synthetic construct
  misc_feature 1..13: note = Sample tag sequence
  source 1..13: mol_type = other DNA
gatccggttgcaa

SEQ ID NO: 131 - DNA, 13 bp, synthetic construct
  misc_feature 1..13: note = Sample tag sequence
  source 1..13: mol_type = other DNA
cgtcaggcttgac

SEQ ID NO: 132 - DNA, 13 bp, synthetic construct
  misc_feature 1..13: note = Sample tag sequence
  source 1..13: mol_type = other DNA
tcggcaaggcgag

SEQ ID NO: 133 - DNA, 13 bp, synthetic construct
  misc_feature 1..13: note = Sample tag sequence
  source 1..13: mol_type = other DNA
gaacggcgaacgc

SEQ ID NO: 134 - DNA, 13 bp, synthetic construct
  misc_feature 1..13: note = Sample tag sequence
  source 1..13: mol_type = other DNA
cctcaagcggact

SEQ ID NO: 135 - DNA, 13 bp, synthetic construct
  misc_feature 1..13: note = Sample tag sequence
  source 1..13: mol_type = other DNA
gaagccagatggt

SEQ ID NO: 136 - DNA, 13 bp, synthetic construct
  misc_feature 1..13: note = Sample tag sequence
  source 1..13: mol_type = other DNA
tgctcataccaat